European Patent Application EP 4 667 015 A1, published December 24, 2025. Title: Vaccine of Lactococcus garvieae of new serotype. Applicant: Kyoritsu Seiyaku Corporation. The sequence listing filed with the application follows.

SEQUENCE LISTING (2 sequences)

SEQ ID NO: 1 - DNA, 256 bp, Lactococcus garvieae
  source 1..256: mol_type = other DNA
acgaaggacttcaagcgcgtttagcacttgcgaatgcgacttcacttgtcttaaaagaagccttgcgcttacttggtgttgaagcacctgaggaaatgtaaattttcaaataaaaaaatagaccagatggtctatttttttatttgtttggtctcacgccttctggccaccaaagtttaatcagcgcttgtgtaccatcattttcataaccttcttctgctaagcgatcataaagctttttcgctcctgctgtggc

SEQ ID NO: 2 - DNA, 258 bp, Lactococcus garvieae
  source 1..258: mol_type = other DNA
acgaaggacttcaagcgcgtttagcacttgcgaatgcgacttcacttgtcttaaaagaagcattgcgcttacttggtgttgaagcacctgaggaaatgtaaattttcaaataaaaaaaatagaccagatggtctattttttttatttgtttggtctcacgccttctggccaccaaagtttaatcagcgcttgtgtaccatcattttcataaccttcttctgctaagcgatcataaagctttttcgctcctgctgtggc